European Patent Application EP 4 563 704 A1, published June 4, 2025. Title: GENE DELIVERY VECTOR FOR DELIVERING HUMAN VEGF RECEPTOR FUSION PROTEIN AND USE THEREOF. Applicant: Shanghai Correge Pharmaceutical Technology Co.,Ltd. The sequence listing filed with the application follows.

SEQUENCE LISTING (11 sequences)

SEQ ID NO: 1 - protein, 103 aa, synthetic construct
SDTGRPFVEMYSEIPEIIHMTEGRELVIPCRVTSPNITVTLKKFPLDTLIPDGKRIIWDSRKGFIISNATYKEIGLLTCEATVNGHLYKTNYLTHRQTNTIID

SEQ ID NO: 2 - protein, 102 aa, synthetic construct
VVLSPSHGIELSVGEKLVLNCTARTELNVGIDFNWEYPSSKHQHKKLVNRDLKTQSGSEMKKFLSTLTIDGVTRSDQGLYTCAASSGLMTKKNSTFVRVHEK

SEQ ID NO: 3 - protein, 226 aa, synthetic construct
DKTHTCPPCPAPELLGGPSVFLFPPKPKDTLYITREPEVTCVVVDVSHEDPEVKFNWYVDGVEVHNAKTKPREEQYNSTYRVVSVLTVLHQDWLNGKEYKCKVSNKALPAPIEKTISKAKGQPREPQVYTLPPSRDELTKNQVSLTCLVKGFYPSDIAVEWESNGQPENNYKTTPPVLDSDGSFFLYSKLTVDKSRWQQGNVFSCSVMHEALHNHYTQKSLSLSPG

SEQ ID NO: 4 - protein, 26 aa, synthetic construct
MVSYWDTGVLLCALLSCLLLTGSSSG

SEQ ID NO: 5 - protein, 457 aa, synthetic construct
MVSYWDTGVLLCALLSCLLLTGSSSGSDTGRPFVEMYSEIPEIIHMTEGRELVIPCRVTSPNITVTLKKFPLDTLIPDGKRIIWDSRKGFIISNATYKEIGLLTCEATVNGHLYKTNYLTHRQTNTIIDVVLSPSHGIELSVGEKLVLNCTARTELNVGIDFNWEYPSSKHQHKKLVNRDLKTQSGSEMKKFLSTLTIDGVTRSDQGLYTCAASSGLMTKKNSTFVRVHEKDKTHTCPPCPAPELLGGPSVFLFPPKPKDTLYITREPEVTCVVVDVSHEDPEVKFNWYVDGVEVHNAKTKPREEQYNSTYRVVSVLTVLHQDWLNGKEYKCKVSNKALPAPIEKTISKAKGQPREPQVYTLPPSRDELTKNQVSLTCLVKGFYPSDIAVEWESNGQPENNYKTTPPVLDSDGSFFLYSKLTVDKSRWQQGNVFSCSVMHEALHNHYTQKSLSLSPG

SEQ ID NO: 6 - protein, 100 aa, synthetic construct
GRPFVEMYSEIPEIIHMTEGRELVIPCRVTSPNITVTLKKFPLDTLIPDGKRIIWDSRKGFIISNATYKEIGLLTCEATVNGHLYKTNYLTHRQTNTIID

SEQ ID NO: 7 - protein, 97 aa, synthetic construct
PFVAFGSGMESLVEATVGERVRIPAKYLGYPPPEIKWYKNGIPLESNHTIKAGHVLTIMEVSERDTGNYTVILTNPISKEKQSHVVSLVVYVPPGPG

SEQ ID NO: 8 - protein, 227 aa, synthetic construct
DKTHTCPLCPAPELLGGPSVFLFPPKPKDTLYITREPEVTCVVVDVSHEDPEVKFNWYVDGVEVHNAKTKPREEQYNSTYRVVSVLTVLHQDWLNGKEYKCKVSNKALPAPIEKTISKAKGQPREPQVYTLPPSRDELTKNQVSLTCLVKGFYPSDIAVEWESNGQPENNYKATPPVLDSDGSFFLYSKLTVDKSRWQQGNVFSCSVMHEALHNHYTQKSLSLSPGK

SEQ ID NO: 9 - protein, 552 aa, synthetic construct
MVSYWDTGVLLCALLSCLLLTGSSSGGRPFVEMYSEIPEIIHMTEGRELVIPCRVTSPNITVTLKKFPLDTLIPDGKRIIWDSRKGFIISNATYKEIGLLTCEATVNGHLYKTNYLTHRQTNTIIDVVLSPSHGIELSVGEKLVLNCTARTELNVGIDFNWEYPSSKHQHKKLVNRDLKTQSGSEMKKFLSTLTIDGVTRSDQGLYTCAASSGLMTKKNSTFVRVHEKPFVAFGSGMESLVEATVGERVRIPAKYLGYPPPEIKWYKNGIPLESNHTIKAGHVLTIMEVSERDTGNYTVILTNPISKEKQSHVVSLVVYVPPGPGDKTHTCPLCPAPELLGGPSVFLFPPKPKDTLYITREPEVTCVVVDVSHEDPEVKFNWYVDGVEVHNAKTKPREEQYNSTYRVVSVLTVLHQDWLNGKEYKCKVSNKALPAPIEKTISKAKGQPREPQVYTLPPSRDELTKNQVSLTCLVKGFYPSDIAVEWESNGQPENNYKATPPVLDSDGSFFLYSKLTVDKSRWQQGNVFSCSVMHEALHNHYTQKSLSLSPGK

SEQ ID NO: 10 - DNA, 1374 bp, synthetic construct
  source 1..1374: mol_type = other DNA
atggtgtcctactgggacacaggcgtgctgttgtgcgccctgctgtcttgtctgctgctgacaggatctagcagcggcagcgatacaggccggccttttgtggaaatgtactctgaaatccccgagatcatccacatgaccgagggcagagagctggtgatcccctgcagagtcacatcccccaacatcaccgtgaccctgaagaaattccccctggataccctgatccctgacggcaagagaatcatctgggatagcagaaaaggctttatcatcagcaacgccacctacaaggaaatcggcctgctgacctgcgaggccactgtgaacggccacctgtacaagacaaactacctgacacacagacagaccaacaccatcattgatgtggtgctctctcctagccacggcatcgagctgtctgtgggcgagaaactggtgctgaactgcaccgctagaaccgagcttaatgtgggaatcgacttcaattgggagtatccatcaagtaagcaccaacacaagaagctggtgaacagggacctgaaaacacagagtggctctgagatgaaaaagttcctgagcaccctgacaatcgacggagttacaagaagcgaccagggcctgtacacctgtgccgccagcagcggcctgatgaccaagaagaatagcacatttgtgcgggtgcacgagaaggacaagacccacacctgcccaccatgtcctgctcctgagctgctgggcggccctagcgtgttcctgttccctcctaagcccaaggataccctgtacatcaccagagagcccgaggtgacctgcgtggtggtcgacgtgtctcatgaagatcctgaggtgaagttcaactggtacgtggacggagttgaagtgcacaatgccaagaccaagcctagagaggaacagtacaacagcacctaccgggtggtcagcgtgctgaccgtcctgcaccaggactggctgaacggcaaggaatacaaatgcaaggtgtccaacaaggccctgcccgcccctatcgagaagacgattagcaaagctaagggacagcctcgggaaccccaggtgtacaccctgcctccaagccgggacgagctgacaaagaaccaggtgtccctgacatgtctggtcaagggcttctacccctctgatatcgccgtggaatgggaaagcaacggccaacctgaaaacaactacaaaacaacccctcctgtgctggacagcgacggcagcttcttcctgtatagcaagctgaccgtggataagagccgctggcagcagggcaacgtgttcagctgcagcgtgatgcacgaggcccttcataatcactacacccagaagtccctgagcctgagccctggctaa

SEQ ID NO: 11 - DNA, 1659 bp, synthetic construct
  source 1..1659: mol_type = other DNA
atggtcagctactgggacaccggggtcctgctgtgcgcgctgctcagctgtctgcttctcacaggatctagttccggaggtagacctttcgtagagatgtacagtgaaatccccgaaattatacacatgactgaaggaagggagctcgtcattccctgccgggttacgtcacctaacatcactgttactttaaaaaagtttccacttgacactttgatccctgatggaaaacgcataatctgggacagtagaaagggcttcatcatatcaaatgcaacgtacaaagaaatagggcttctgacctgtgaagcaacagtcaatgggcatttgtataagacaaactatctcacacatcgacaaaccaatacaatcatagatgtggttctgagtccgtctcatggaattgaactatctgttggagaaaagcttgtcttaaattgtacagcaagaactgaactaaatgtggggattgacttcaactgggaatacccttcttcgaagcatcagcataagaaacttgtaaaccgagacctaaaaacccagtctgggagtgagatgaagaaatttttgagcaccttaactatagatggtgtaacccggagtgaccaaggattgtacacctgtgcagcatccagtgggctgatgaccaagaagaacagcacatttgtcagggtccatgaaaaaccttttgttgcttttggaagtggcatggaatctctggtggaagccacggtgggggagcgtgtcagaatccctgcgaagtaccttggttacccacccccagaaataaaatggtataaaaatggaataccccttgagtccaatcacacaattaaagcggggcatgtactgacgattatggaagtgagtgaaagagacacaggaaattacactgtcatccttaccaatcccatttcaaaggagaagcagagccatgtggtctctctggttgtgtatgtcccaccgggcccgggcgacaaaactcacacatgcccactgtgcccagcacctgaactcctggggggaccgtcagtcttcctcttccccccaaaacccaaggacaccctctacatcacccgggagcctgaggtcacatgcgtggtggtggacgtgagccacgaagaccctgaggtcaagttcaactggtacgtggacggcgtggaggtgcataatgccaagacaaagccgcgggaggagcagtacaacagcacgtaccgtgtggtcagcgtcctcaccgtcctgcaccaggactggctgaatggcaaggagtacaagtgcaaggtctccaacaaagccctcccagcccccatcgagaaaaccatctccaaagccaaagggcagccccgagaaccacaggtgtacaccctgcccccatcccgggatgagctgaccaagaaccaggtcagcctgacctgcctagtcaaaggcttctatcccagcgacatcgccgtggagtgggagagcaatgggcagccggagaacaactacaaggccacgcctcccgtgctggactccgacggctccttcttcctctacagcaagctcaccgtggacaagagcaggtggcagcaggggaacgtcttctcatgctccgtgatgcatgaggctctgcacaaccactacacgcagaagagcctctccctgtctccgggtaaatga